European Patent Application EP 4 249 593 A1, published September 27, 2023. Title: aroG Aldolase Variant and Method for Producing Branched-Chain Amino Acids Using the Same. Applicant: CJ CheilJedang Corporation. The sequence listing filed with the application follows.

SEQUENCE LISTING (63 sequences)

SEQ ID NO: 1 - protein, 466 aa, Unknown
  aroG_WT
MNRGVSWTVDIPKEVLPDLPPLPEGMQQQFEDTISRDAKQQPTWDRAQAENVRKILESVPPIVVAPEVLELKQKLADVANGKAFLLQGGDCAETFESNTEPHIRANVKTLLQMAVVLTYGASTPVIKMARIAGQYAKPRSSDLDGNGLPNYRGDIVNGVEATPEARRHDPARMIRAYANASAAMNLVRALTSSGTADLYRLSEWNREFVANSPAGARYEALAREIDSGLRFMEACGVSDESLRAADIYCSHEALLVDYERSMLRLATDEEGNEELYDLSAHQLWIGERTRGMDDFHVNFASMISNPIGIKIGPGITPEEAVAYADKLDPNFEPGRLTIVARMGHDKVRSVLPGVIQAVEASGHKVIWQSDPMHGNTFTASNGYKTRHFDKVIDEVQGFFEVHRALGTHPGGIHIEFTGEDVTECLGGAEDITDVDLPGRYESACDPRLNTQQSLELAFLVAEMLRN

SEQ ID NO: 2 - DNA, 1401 bp, Unknown
  aroG_WT
atgaataggggtgtgagttggacagttgatatccctaaagaagttctccctgatttgccaccattgccagaaggcatgcagcagcagttcgaggacaccatttcccgtgacgctaagcagcaacctacgtgggatcgtgcacaggcagaaaacgtgcgcaagatccttgagtcggttcctccaatcgttgttgcccctgaggtacttgagctgaagcagaagcttgctgatgttgccaacggtaaggccttcctcttgcagggtggtgactgtgcggaaactttcgagtcaaacactgagccgcacattcgcgccaacgtaaagactctgctgcagatggcagttgttttgacctacggtgcatccactcctgtgatcaagatggctcgtattgctggtcagtacgcaaagcctcgctcttctgatctggatggaaatggtctgccaaactaccgtggcgatatcgtcaacggtgtggaggcaaccccagaggctcgtcgccacgatcctgcccgcatgatccgtgcttacgctaacgcttctgctgcgatgaacttggtgcgcgcgctcaccagctctggcaccgctgatctttaccgtctcagcgagtggaaccgcgagttcgttgcgaactccccagctggtgcacgctacgaggctcttgctcgtgagatcgactccggtctgcgcttcatggaagcatgtggcgtgtccgatgagtccctgcgtgctgcagatatctactgctcccacgaggctttgctggtggattacgagcgttccatgctgcgtcttgcaaccgatgaggaaggcaacgaggaactttacgatctttcagctcaccagctgtggatcggcgagcgcacccgtggcatggatgatttccatgtgaacttcgcatccatgatctctaacccaatcggcatcaagattggtcctggtatcacccctgaagaggctgttgcatacgctgacaagctcgatccgaacttcgagcctggccgtttgaccatcgttgctcgcatgggccacgacaaggttcgctccgtacttcctggtgttatccaggctgttgaggcatccggacacaaggttatttggcagtccgatccgatgcacggcaacactttcaccgcatccaatggctacaagacccgtcacttcgacaaggttatcgatgaggtccagggcttcttcgaggtccaccgcgcattgggcacccacccaggcggaatccacattgagttcactggtgaagatgtcaccgagtgcctcggtggcgctgaagacatcaccgatgttgatctgccaggccgctacgagtccgcatgcgatcctcgcctgaacactcagcagtctttggagttggctttcctcgttgcagaaatgctgcgtaactaa

SEQ ID NO: 3 - protein, 466 aa, Artificial Sequence
  aroG_R217A
MNRGVSWTVDIPKEVLPDLPPLPEGMQQQFEDTISRDAKQQPTWDRAQAENVRKILESVPPIVVAPEVLELKQKLADVANGKAFLLQGGDCAETFESNTEPHIRANVKTLLQMAVVLTYGASTPVIKMARIAGQYAKPRSSDLDGNGLPNYRGDIVNGVEATPEARRHDPARMIRAYANASAAMNLVRALTSSGTADLYRLSEWNREFVANSPAGAAYEALAREIDSGLRFMEACGVSDESLRAADIYCSHEALLVDYERSMLRLATDEEGNEELYDLSAHQLWIGERTRGMDDFHVNFASMISNPIGIKIGPGITPEEAVAYADKLDPNFEPGRLTIVARMGHDKVRSVLPGVIQAVEASGHKVIWQSDPMHGNTFTASNGYKTRHFDKVIDEVQGFFEVHRALGTHPGGIHIEFTGEDVTECLGGAEDITDVDLPGRYESACDPRLNTQQSLELAFLVAEMLRN

SEQ ID NO: 4 - DNA, 1401 bp, Artificial Sequence
  aroG_R217A_nt
atgaataggggtgtgagttggacagttgatatccctaaagaagttctccctgatttgccaccattgccagaaggcatgcagcagcagttcgaggacaccatttcccgtgacgctaagcagcaacctacgtgggatcgtgcacaggcagaaaacgtgcgcaagatccttgagtcggttcctccaatcgttgttgcccctgaggtacttgagctgaagcagaagcttgctgatgttgccaacggtaaggccttcctcttgcagggtggtgactgtgcggaaactttcgagtcaaacactgagccgcacattcgcgccaacgtaaagactctgctgcagatggcagttgttttgacctacggtgcatccactcctgtgatcaagatggctcgtattgctggtcagtacgcaaagcctcgctcttctgatctggatggaaatggtctgccaaactaccgtggcgatatcgtcaacggtgtggaggcaaccccagaggctcgtcgccacgatcctgcccgcatgatccgtgcttacgctaacgcttctgctgcgatgaacttggtgcgcgcgctcaccagctctggcaccgctgatctttaccgtctcagcgagtggaaccgcgagttcgttgcgaactccccagctggtgcagcgtacgaggctcttgctcgtgagatcgactccggtctgcgcttcatggaagcatgtggcgtgtccgatgagtccctgcgtgctgcagatatctactgctcccacgaggctttgctggtggattacgagcgttccatgctgcgtcttgcaaccgatgaggaaggcaacgaggaactttacgatctttcagctcaccagctgtggatcggcgagcgcacccgtggcatggatgatttccatgtgaacttcgcatccatgatctctaacccaatcggcatcaagattggtcctggtatcacccctgaagaggctgttgcatacgctgacaagctcgatccgaacttcgagcctggccgtttgaccatcgttgctcgcatgggccacgacaaggttcgctccgtacttcctggtgttatccaggctgttgaggcatccggacacaaggttatttggcagtccgatccgatgcacggcaacactttcaccgcatccaatggctacaagacccgtcacttcgacaaggttatcgatgaggtccagggcttcttcgaggtccaccgcgcattgggcacccacccaggcggaatccacattgagttcactggtgaagatgtcaccgagtgcctcggtggcgctgaagacatcaccgatgttgatctgccaggccgctacgagtccgcatgcgatcctcgcctgaacactcagcagtctttggagttggctttcctcgttgcagaaatgctgcgtaactaa

SEQ ID NO: 5 - protein, 466 aa, Artificial Sequence
  aroG_K310A
MNRGVSWTVDIPKEVLPDLPPLPEGMQQQFEDTISRDAKQQPTWDRAQAENVRKILESVPPIVVAPEVLELKQKLADVANGKAFLLQGGDCAETFESNTEPHIRANVKTLLQMAVVLTYGASTPVIKMARIAGQYAKPRSSDLDGNGLPNYRGDIVNGVEATPEARRHDPARMIRAYANASAAMNLVRALTSSGTADLYRLSEWNREFVANSPAGARYEALAREIDSGLRFMEACGVSDESLRAADIYCSHEALLVDYERSMLRLATDEEGNEELYDLSAHQLWIGERTRGMDDFHVNFASMISNPIGIAIGPGITPEEAVAYADKLDPNFEPGRLTIVARMGHDKVRSVLPGVIQAVEASGHKVIWQSDPMHGNTFTASNGYKTRHFDKVIDEVQGFFEVHRALGTHPGGIHIEFTGEDVTECLGGAEDITDVDLPGRYESACDPRLNTQQSLELAFLVAEMLRN

SEQ ID NO: 6 - DNA, 1401 bp, Artificial Sequence
  aroG_K310A_nt
atgaataggggtgtgagttggacagttgatatccctaaagaagttctccctgatttgccaccattgccagaaggcatgcagcagcagttcgaggacaccatttcccgtgacgctaagcagcaacctacgtgggatcgtgcacaggcagaaaacgtgcgcaagatccttgagtcggttcctccaatcgttgttgcccctgaggtacttgagctgaagcagaagcttgctgatgttgccaacggtaaggccttcctcttgcagggtggtgactgtgcggaaactttcgagtcaaacactgagccgcacattcgcgccaacgtaaagactctgctgcagatggcagttgttttgacctacggtgcatccactcctgtgatcaagatggctcgtattgctggtcagtacgcaaagcctcgctcttctgatctggatggaaatggtctgccaaactaccgtggcgatatcgtcaacggtgtggaggcaaccccagaggctcgtcgccacgatcctgcccgcatgatccgtgcttacgctaacgcttctgctgcgatgaacttggtgcgcgcgctcaccagctctggcaccgctgatctttaccgtctcagcgagtggaaccgcgagttcgttgcgaactccccagctggtgcacgctacgaggctcttgctcgtgagatcgactccggtctgcgcttcatggaagcatgtggcgtgtccgatgagtccctgcgtgctgcagatatctactgctcccacgaggctttgctggtggattacgagcgttccatgctgcgtcttgcaaccgatgaggaaggcaacgaggaactttacgatctttcagctcaccagctgtggatcggcgagcgcacccgtggcatggatgatttccatgtgaacttcgcatccatgatctctaacccaatcggcatcgcgattggtcctggtatcacccctgaagaggctgttgcatacgctgacaagctcgatccgaacttcgagcctggccgtttgaccatcgttgctcgcatgggccacgacaaggttcgctccgtacttcctggtgttatccaggctgttgaggcatccggacacaaggttatttggcagtccgatccgatgcacggcaacactttcaccgcatccaatggctacaagacccgtcacttcgacaaggttatcgatgaggtccagggcttcttcgaggtccaccgcgcattgggcacccacccaggcggaatccacattgagttcactggtgaagatgtcaccgagtgcctcggtggcgctgaagacatcaccgatgttgatctgccaggccgctacgagtccgcatgcgatcctcgcctgaacactcagcagtctttggagttggctttcctcgttgcagaaatgctgcgtaactaa

SEQ ID NO: 7 - protein, 466 aa, Artificial Sequence
  aroG_R403A
MNRGVSWTVDIPKEVLPDLPPLPEGMQQQFEDTISRDAKQQPTWDRAQAENVRKILESVPPIVVAPEVLELKQKLADVANGKAFLLQGGDCAETFESNTEPHIRANVKTLLQMAVVLTYGASTPVIKMARIAGQYAKPRSSDLDGNGLPNYRGDIVNGVEATPEARRHDPARMIRAYANASAAMNLVRALTSSGTADLYRLSEWNREFVANSPAGARYEALAREIDSGLRFMEACGVSDESLRAADIYCSHEALLVDYERSMLRLATDEEGNEELYDLSAHQLWIGERTRGMDDFHVNFASMISNPIGIKIGPGITPEEAVAYADKLDPNFEPGRLTIVARMGHDKVRSVLPGVIQAVEASGHKVIWQSDPMHGNTFTASNGYKTRHFDKVIDEVQGFFEVHAALGTHPGGIHIEFTGEDVTECLGGAEDITDVDLPGRYESACDPRLNTQQSLELAFLVAEMLRN

SEQ ID NO: 8 - DNA, 1401 bp, Artificial Sequence
  aroG_R403A_nt
atgaataggggtgtgagttggacagttgatatccctaaagaagttctccctgatttgccaccattgccagaaggcatgcagcagcagttcgaggacaccatttcccgtgacgctaagcagcaacctacgtgggatcgtgcacaggcagaaaacgtgcgcaagatccttgagtcggttcctccaatcgttgttgcccctgaggtacttgagctgaagcagaagcttgctgatgttgccaacggtaaggccttcctcttgcagggtggtgactgtgcggaaactttcgagtcaaacactgagccgcacattcgcgccaacgtaaagactctgctgcagatggcagttgttttgacctacggtgcatccactcctgtgatcaagatggctcgtattgctggtcagtacgcaaagcctcgctcttctgatctggatggaaatggtctgccaaactaccgtggcgatatcgtcaacggtgtggaggcaaccccagaggctcgtcgccacgatcctgcccgcatgatccgtgcttacgctaacgcttctgctgcgatgaacttggtgcgcgcgctcaccagctctggcaccgctgatctttaccgtctcagcgagtggaaccgcgagttcgttgcgaactccccagctggtgcacgctacgaggctcttgctcgtgagatcgactccggtctgcgcttcatggaagcatgtggcgtgtccgatgagtccctgcgtgctgcagatatctactgctcccacgaggctttgctggtggattacgagcgttccatgctgcgtcttgcaaccgatgaggaaggcaacgaggaactttacgatctttcagctcaccagctgtggatcggcgagcgcacccgtggcatggatgatttccatgtgaacttcgcatccatgatctctaacccaatcggcatcaagattggtcctggtatcacccctgaagaggctgttgcatacgctgacaagctcgatccgaacttcgagcctggccgtttgaccatcgttgctcgcatgggccacgacaaggttcgctccgtacttcctggtgttatccaggctgttgaggcatccggacacaaggttatttggcagtccgatccgatgcacggcaacactttcaccgcatccaatggctacaagacccgtcacttcgacaaggttatcgatgaggtccagggcttcttcgaggtccacgcggcattgggcacccacccaggcggaatccacattgagttcactggtgaagatgtcaccgagtgcctcggtggcgctgaagacatcaccgatgttgatctgccaggccgctacgagtccgcatgcgatcctcgcctgaacactcagcagtctttggagttggctttcctcgttgcagaaatgctgcgtaactaa

SEQ ID NO: 9 - protein, 466 aa, Artificial Sequence
  aroG_E462A
MNRGVSWTVDIPKEVLPDLPPLPEGMQQQFEDTISRDAKQQPTWDRAQAENVRKILESVPPIVVAPEVLELKQKLADVANGKAFLLQGGDCAETFESNTEPHIRANVKTLLQMAVVLTYGASTPVIKMARIAGQYAKPRSSDLDGNGLPNYRGDIVNGVEATPEARRHDPARMIRAYANASAAMNLVRALTSSGTADLYRLSEWNREFVANSPAGARYEALAREIDSGLRFMEACGVSDESLRAADIYCSHEALLVDYERSMLRLATDEEGNEELYDLSAHQLWIGERTRGMDDFHVNFASMISNPIGIKIGPGITPEEAVAYADKLDPNFEPGRLTIVARMGHDKVRSVLPGVIQAVEASGHKVIWQSDPMHGNTFTASNGYKTRHFDKVIDEVQGFFEVHRALGTHPGGIHIEFTGEDVTECLGGAEDITDVDLPGRYESACDPRLNTQQSLELAFLVAAMLRN

SEQ ID NO: 10 - DNA, 1401 bp, Artificial Sequence
  aroG_E462A_nt
atgaataggggtgtgagttggacagttgatatccctaaagaagttctccctgatttgccaccattgccagaaggcatgcagcagcagttcgaggacaccatttcccgtgacgctaagcagcaacctacgtgggatcgtgcacaggcagaaaacgtgcgcaagatccttgagtcggttcctccaatcgttgttgcccctgaggtacttgagctgaagcagaagcttgctgatgttgccaacggtaaggccttcctcttgcagggtggtgactgtgcggaaactttcgagtcaaacactgagccgcacattcgcgccaacgtaaagactctgctgcagatggcagttgttttgacctacggtgcatccactcctgtgatcaagatggctcgtattgctggtcagtacgcaaagcctcgctcttctgatctggatggaaatggtctgccaaactaccgtggcgatatcgtcaacggtgtggaggcaaccccagaggctcgtcgccacgatcctgcccgcatgatccgtgcttacgctaacgcttctgctgcgatgaacttggtgcgcgcgctcaccagctctggcaccgctgatctttaccgtctcagcgagtggaaccgcgagttcgttgcgaactccccagctggtgcacgctacgaggctcttgctcgtgagatcgactccggtctgcgcttcatggaagcatgtggcgtgtccgatgagtccctgcgtgctgcagatatctactgctcccacgaggctttgctggtggattacgagcgttccatgctgcgtcttgcaaccgatgaggaaggcaacgaggaactttacgatctttcagctcaccagctgtggatcggcgagcgcacccgtggcatggatgatttccatgtgaacttcgcatccatgatctctaacccaatcggcatcaagattggtcctggtatcacccctgaagaggctgttgcatacgctgacaagctcgatccgaacttcgagcctggccgtttgaccatcgttgctcgcatgggccacgacaaggttcgctccgtacttcctggtgttatccaggctgttgaggcatccggacacaaggttatttggcagtccgatccgatgcacggcaacactttcaccgcatccaatggctacaagacccgtcacttcgacaaggttatcgatgaggtccagggcttcttcgaggtccaccgcgcattgggcacccacccaggcggaatccacattgagttcactggtgaagatgtcaccgagtgcctcggtggcgctgaagacatcaccgatgttgatctgccaggccgctacgagtccgcatgcgatcctcgcctgaacactcagcagtctttggagttggctttcctcgttgcagcgatgctgcgtaactaa

SEQ ID NO: 11 - DNA, 20 bp, Artificial Sequence
  primer
tgatgcgcgtcataatttag

SEQ ID NO: 12 - DNA, 20 bp, Artificial Sequence
  primer
ctcatctctgactggacgtg

SEQ ID NO: 13 - DNA, 41 bp, Artificial Sequence
  primer
gtgaattcgagctcggtacccagttgaatgctaccaacttg

SEQ ID NO: 14 - DNA, 35 bp, Artificial Sequence
  primer
cacgagcaagagcctcgtacgctgcaccagctggg

SEQ ID NO: 15 - DNA, 40 bp, Artificial Sequence
  primer
ggtcgactctagaggatccccgctgttattactgtgcctg

SEQ ID NO: 16 - DNA, 39 bp, Artificial Sequence
  primer
gaactccccagctggtgcagcgtacgaggctcttgctcg

SEQ ID NO: 17 - DNA, 39 bp, Artificial Sequence
  primer
gggtgataccaggaccaatcgcgatgccgattgggttag

SEQ ID NO: 18 - DNA, 39 bp, Artificial Sequence
  primer
ctctaacccaatcggcatcgcgattggtcctggtatcac

SEQ ID NO: 19 - DNA, 38 bp, Artificial Sequence
  primer
ctgggtgggtgcccaatgccgcgtggacctcgaagaag

SEQ ID NO: 20 - DNA, 37 bp, Artificial Sequence
  primer
gggcttcttcgaggtccacgcggcattgggcacccac

SEQ ID NO: 21 - DNA, 38 bp, Artificial Sequence
  primer
aagcttagttacgcagcatcgctgcaacgaggaaagcc

SEQ ID NO: 22 - DNA, 39 bp, Artificial Sequence
  primer
gttggctttcctcgttgcagcgatgctgcgtaactaagc

SEQ ID NO: 23 - protein, 466 aa, Artificial Sequence
  aroG_R217A+K310A+E462A
MNRGVSWTVDIPKEVLPDLPPLPEGMQQQFEDTISRDAKQQPTWDRAQAENVRKILESVPPIVVAPEVLELKQKLADVANGKAFLLQGGDCAETFESNTEPHIRANVKTLLQMAVVLTYGASTPVIKMARIAGQYAKPRSSDLDGNGLPNYRGDIVNGVEATPEARRHDPARMIRAYANASAAMNLVRALTSSGTADLYRLSEWNREFVANSPAGAAYEALAREIDSGLRFMEACGVSDESLRAADIYCSHEALLVDYERSMLRLATDEEGNEELYDLSAHQLWIGERTRGMDDFHVNFASMISNPIGIAIGPGITPEEAVAYADKLDPNFEPGRLTIVARMGHDKVRSVLPGVIQAVEASGHKVIWQSDPMHGNTFTASNGYKTRHFDKVIDEVQGFFEVHRALGTHPGGIHIEFTGEDVTECLGGAEDITDVDLPGRYESACDPRLNTQQSLELAFLVAAMLRN

SEQ ID NO: 24 - DNA, 1401 bp, Artificial Sequence
  aroG_R217A+K310A+E462A_nt
atgaataggggtgtgagttggacagttgatatccctaaagaagttctccctgatttgccaccattgccagaaggcatgcagcagcagttcgaggacaccatttcccgtgacgctaagcagcaacctacgtgggatcgtgcacaggcagaaaacgtgcgcaagatccttgagtcggttcctccaatcgttgttgcccctgaggtacttgagctgaagcagaagcttgctgatgttgccaacggtaaggccttcctcttgcagggtggtgactgtgcggaaactttcgagtcaaacactgagccgcacattcgcgccaacgtaaagactctgctgcagatggcagttgttttgacctacggtgcatccactcctgtgatcaagatggctcgtattgctggtcagtacgcaaagcctcgctcttctgatctggatggaaatggtctgccaaactaccgtggcgatatcgtcaacggtgtggaggcaaccccagaggctcgtcgccacgatcctgcccgcatgatccgtgcttacgctaacgcttctgctgcgatgaacttggtgcgcgcgctcaccagctctggcaccgctgatctttaccgtctcagcgagtggaaccgcgagttcgttgcgaactccccagctggtgcagcgtacgaggctcttgctcgtgagatcgactccggtctgcgcttcatggaagcatgtggcgtgtccgatgagtccctgcgtgctgcagatatctactgctcccacgaggctttgctggtggattacgagcgttccatgctgcgtcttgcaaccgatgaggaaggcaacgaggaactttacgatctttcagctcaccagctgtggatcggcgagcgcacccgtggcatggatgatttccatgtgaacttcgcatccatgatctctaacccaatcggcatcgcgattggtcctggtatcacccctgaagaggctgttgcatacgctgacaagctcgatccgaacttcgagcctggccgtttgaccatcgttgctcgcatgggccacgacaaggttcgctccgtacttcctggtgttatccaggctgttgaggcatccggacacaaggttatttggcagtccgatccgatgcacggcaacactttcaccgcatccaatggctacaagacccgtcacttcgacaaggttatcgatgaggtccagggcttcttcgaggtccaccgcgcattgggcacccacccaggcggaatccacattgagttcactggtgaagatgtcaccgagtgcctcggtggcgctgaagacatcaccgatgttgatctgccaggccgctacgagtccgcatgcgatcctcgcctgaacactcagcagtctttggagttggctttcctcgttgcagcgatgctgcgtaactaa

SEQ ID NO: 25 - protein, 466 aa, Artificial Sequence
  aroG_R217A+K310A+R403A+E462A
MNRGVSWTVDIPKEVLPDLPPLPEGMQQQFEDTISRDAKQQPTWDRAQAENVRKILESVPPIVVAPEVLELKQKLADVANGKAFLLQGGDCAETFESNTEPHIRANVKTLLQMAVVLTYGASTPVIKMARIAGQYAKPRSSDLDGNGLPNYRGDIVNGVEATPEARRHDPARMIRAYANASAAMNLVRALTSSGTADLYRLSEWNREFVANSPAGAAYEALAREIDSGLRFMEACGVSDESLRAADIYCSHEALLVDYERSMLRLATDEEGNEELYDLSAHQLWIGERTRGMDDFHVNFASMISNPIGIAIGPGITPEEAVAYADKLDPNFEPGRLTIVARMGHDKVRSVLPGVIQAVEASGHKVIWQSDPMHGNTFTASNGYKTRHFDKVIDEVQGFFEVHAALGTHPGGIHIEFTGEDVTECLGGAEDITDVDLPGRYESACDPRLNTQQSLELAFLVAAMLRN

SEQ ID NO: 26 - DNA, 1401 bp, Artificial Sequence
  aroG_R217A+K310A+R403A+E462A_nt
atgaataggggtgtgagttggacagttgatatccctaaagaagttctccctgatttgccaccattgccagaaggcatgcagcagcagttcgaggacaccatttcccgtgacgctaagcagcaacctacgtgggatcgtgcacaggcagaaaacgtgcgcaagatccttgagtcggttcctccaatcgttgttgcccctgaggtacttgagctgaagcagaagcttgctgatgttgccaacggtaaggccttcctcttgcagggtggtgactgtgcggaaactttcgagtcaaacactgagccgcacattcgcgccaacgtaaagactctgctgcagatggcagttgttttgacctacggtgcatccactcctgtgatcaagatggctcgtattgctggtcagtacgcaaagcctcgctcttctgatctggatggaaatggtctgccaaactaccgtggcgatatcgtcaacggtgtggaggcaaccccagaggctcgtcgccacgatcctgcccgcatgatccgtgcttacgctaacgcttctgctgcgatgaacttggtgcgcgcgctcaccagctctggcaccgctgatctttaccgtctcagcgagtggaaccgcgagttcgttgcgaactccccagctggtgcagcgtacgaggctcttgctcgtgagatcgactccggtctgcgcttcatggaagcatgtggcgtgtccgatgagtccctgcgtgctgcagatatctactgctcccacgaggctttgctggtggattacgagcgttccatgctgcgtcttgcaaccgatgaggaaggcaacgaggaactttacgatctttcagctcaccagctgtggatcggcgagcgcacccgtggcatggatgatttccatgtgaacttcgcatccatgatctctaacccaatcggcatcgcgattggtcctggtatcacccctgaagaggctgttgcatacgctgacaagctcgatccgaacttcgagcctggccgtttgaccatcgttgctcgcatgggccacgacaaggttcgctccgtacttcctggtgttatccaggctgttgaggcatccggacacaaggttatttggcagtccgatccgatgcacggcaacactttcaccgcatccaatggctacaagacccgtcacttcgacaaggttatcgatgaggtccagggcttcttcgaggtccacgcggcattgggcacccacccaggcggaatccacattgagttcactggtgaagatgtcaccgagtgcctcggtggcgctgaagacatcaccgatgttgatctgccaggccgctacgagtccgcatgcgatcctcgcctgaacactcagcagtctttggagttggctttcctcgttgcagcgatgctgcgtaactaa

SEQ ID NO: 27 - DNA, 21 bp, Artificial Sequence
  primer
tatgcttcaccacatgacttc

SEQ ID NO: 28 - DNA, 23 bp, Artificial Sequence
  primer
aaatcatttgagaaaactcgagg

SEQ ID NO: 29 - DNA, 19 bp, Artificial Sequence
  primer
gtcacccgatcgtctgaag

SEQ ID NO: 30 - DNA, 18 bp, Artificial Sequence
  primer
gtcttaaaaccggttgat

SEQ ID NO: 31 - DNA, 19 bp, Artificial Sequence
  primer
caatgctggctgcgtacgc

SEQ ID NO: 32 - DNA, 20 bp, Artificial Sequence
  primer
ctcctcgcgaggaaccaact

SEQ ID NO: 33 - DNA, 35 bp, Artificial Sequence
  primer
tcgagctcggtaccccgcttttgcactcatcgagc

SEQ ID NO: 34 - DNA, 23 bp, Artificial Sequence
  primer
cacgatcagatgtgcatcatcat

SEQ ID NO: 35 - DNA, 23 bp, Artificial Sequence
  primer
atgatgatgcacatctgatcgtg

SEQ ID NO: 36 - DNA, 35 bp, Artificial Sequence
  primer
ctctagaggatccccgagcatcttccaaaaccttg

SEQ ID NO: 37 - DNA, 35 bp, Artificial Sequence
  primer
tcgagctcggtacccatgagtgaaacatacgtgtc

SEQ ID NO: 38 - DNA, 39 bp, Artificial Sequence
  primer
gcgcttgaggtactctgccagcgcgatgtcatcatccgg

SEQ ID NO: 39 - DNA, 39 bp, Artificial Sequence
  primer
ccggatgatgacatcgcgctggcagagtacctcaagcgc

SEQ ID NO: 40 - DNA, 34 bp, Artificial Sequence
  primer
ctctagaggatcccccgtcaccgacacctccaca

SEQ ID NO: 41 - protein, 437 aa, Artificial Sequence
  gltA_M312I
MFERDIVATDNNKAVLHYPGGEFEMDIIEASEGNNGVVLGKMLSETGLITFDPGYVSTGSTESKITYIDGDAGILRYRGYDIADLAENATFNEVSYLLINGELPTPDELHKFNDEIRHHTLLDEDFKSQFNVFPRDAHPMATLASSVNILSTYYQDQLNPLDEAQLDKATVRLMAKVPMLAAYAHRARKGAPYMYPDNSLNARENFLRMMFGYPTEPYEIDPIMVKALDKLLILHADHEQNCSTSTVRMIGSAQANMFVSIAGGINALSGPLHGGANQAVLEMLEDIKSNHGGDATEFMNKVKNKEDGVRLIGFGHRVYKNYDPRAAIVKETAHEILEHLGGDDLLDLAIKLEEIALADDYFISRKLYPNVDFYTGLIYRAMGFPTDFFTVLFAIGRLPGWIAHYREQLGAAGNKINRPRQVYTGNESRKLVPREER

SEQ ID NO: 42 - DNA, 1314 bp, Artificial Sequence
  gltA_M312I_nt
atgtttgaaagggatatcgtggctactgataacaacaaggctgtcctgcactaccccggtggcgagttcgaaatggacatcatcgaggcttctgagggtaacaacggtgttgtcctgggcaagatgctgtctgagactggactgatcacttttgacccaggttatgtgagcactggctccaccgagtcgaagatcacctacatcgatggcgatgcgggaatcctgcgttaccgcggctatgacatcgctgatctggctgagaatgccaccttcaacgaggtttcttacctacttatcaacggtgagctaccaaccccagatgagcttcacaagtttaacgacgagattcgccaccacacccttctggacgaggacttcaagtcccagttcaacgtgttcccacgcgacgctcacccaatggcaaccttggcttcctcggttaacattttgtctacctactaccaggaccagctgaacccactcgatgaggcacagcttgataaggcaaccgttcgcctcatggcaaaggttccaatgctggctgcgtacgcacaccgcgcacgcaagggtgctccttacatgtacccagacaactccctcaatgcgcgtgagaacttcctgcgcatgatgttcggttacccaaccgagccatacgagatcgacccaatcatggtcaaggctctggacaagctgctcatcctgcacgctgaccacgagcagaactgctccacctccaccgttcgtatgatcggttccgcacaggccaacatgtttgtctccatcgctggtggcatcaacgctctgtccggcccactgcacggtggcgcaaaccaggctgttctggagatgctcgaagacatcaagagcaaccacggtggcgacgcaaccgagttcatgaacaaggtcaagaacaaggaagacggcgtccgcctcatcggcttcggacaccgcgtttacaagaactacgatccacgtgcagcaatcgtcaaggagaccgcacacgagatcctcgagcacctcggtggcgacgatcttctggatctggcaatcaagctggaagaaattgcactggctgatgattacttcatctcccgcaagctctacccgaacgtagacttctacaccggcctgatctaccgcgcaatgggcttcccaactgacttcttcaccgtattgttcgcaatcggtcgtctgccaggatggatcgctcactaccgcgagcagctcggtgcagcaggcaacaagatcaaccgcccacgccaggtctacaccggcaacgaatcccgcaagttggttcctcgcgaggagcgctaa

SEQ ID NO: 43 - DNA, 42 bp, Artificial Sequence
  gltA M312I Up F
gtgaattcgagctcggtacccgcgggaatcctgcgttaccgc

SEQ ID NO: 44 - DNA, 42 bp, Artificial Sequence
  gltA M312I Up R
tgtaaacgcggtgtccgaagccgatgaggcggacgccgtctt

SEQ ID NO: 45 - DNA, 42 bp, Artificial Sequence
  gltA M312I Down F
aagacggcgtccgcctcatcggcttcggacaccgcgtttaca

SEQ ID NO: 46 - DNA, 42 bp, Artificial Sequence
  gltA M312I Down R
ggtcgactctagaggatccccttagcgctcctcgcgaggaac

SEQ ID NO: 47 - protein, 436 aa, Unknown
  ilvA_WT
MSETYVSEKSPGVMASGAELIRAADIQTAQARISSVIAPTPLQYCPRLSEETGAEIYLKREDLQDVRSYKIRGALNSGAQLTQEQRDAGIVAASAGNHAQGVAYVCKSLGVQGRIYVPVQTPKQKRDRIMVHGGEFVSLVVTGNNFDEASAAAHEDAERTGATLIEPFDARNTVIGQGTVAAEILSQLTSMGKSADHVMVPVGGGGLLAGVVSYMADMAPRTAIVGIEPAGAASMQAALHNGGPITLETVDPFVDGAAVKRVGDLNYTIVEKNQGRVHMMSATEGAVCTEMLDLYQNEGIIAEPAGALSIAGLKEMSFAPGSVVVCIISGGNNDVLRYAEIAERSLVHRGLKHYFLVNFPQKPGQLRHFLEDILGPDDDITLFEYLKRNNRETGTALVGIHLSEASGLDSLLERMEESAIDSRRLEPGTPEYEYLT

SEQ ID NO: 48 - DNA, 1311 bp, Unknown
  ilvA_WT_nt
atgagtgaaacatacgtgtctgagaaaagtccaggagtgatggctagcggagcggagctgattcgtgccgccgacattcaaacggcgcaggcacgaatttcctccgtcattgcaccaactccattgcagtattgccctcgtctttctgaggaaaccggagcggaaatctaccttaagcgtgaggatctgcaggatgttcgttcctacaagatccgcggtgcgctgaactctggagcgcagctcacccaagagcagcgcgatgcaggtatcgttgccgcatctgcaggtaaccatgcccagggcgtggcctatgtgtgcaagtccttgggcgttcagggacgcatctatgttcctgtgcagactccaaagcaaaagcgtgaccgcatcatggttcacggcggagagtttgtctccttggtggtcactggcaataacttcgacgaagcatcggctgcagcgcatgaagatgcagagcgcaccggcgcaacgctgatcgagcctttcgatgctcgcaacaccgtcatcggtcagggcaccgtggctgctgagatcttgtcgcagctgacttccatgggcaagagtgcagatcacgtgatggttccagtcggcggtggcggacttcttgcaggtgtggtcagctacatggctgatatggcacctcgcactgcgatcgttggtatcgaaccagcgggagcagcatccatgcaggctgcattgcacaatggtggaccaatcactttggagactgttgatccctttgtggacggcgcagcagtcaaacgtgtcggagatctcaactacaccatcgtggagaagaaccagggtcgcgtgcacatgatgagcgcgaccgagggcgctgtgtgtactgagatgctcgatctttaccaaaacgaaggcatcatcgcggagcctgctggcgcgctgtctatcgctgggttgaaggaaatgtcctttgcacctggttctgtcgtggtgtgcatcatctctggtggcaacaacgatgtgctgcgttatgcggaaatcgctgagcgctccttggtgcaccgcggtttgaagcactacttcttggtgaacttcccgcaaaagcctggtcagttgcgtcacttcctggaagatatcctgggaccggatgatgacatcacgctgtttgagtacctcaagcgcaacaaccgtgagaccggtactgcgttggtgggtattcacttgagtgaagcatcaggattggattctttgctggaacgtatggaggaatcggcaattgattcccgtcgcctcgagccgggcacccctgagtacgaatacttgacctaa

SEQ ID NO: 49 - DNA, 26 bp, Artificial Sequence
  primer
ggatccgactgagcctgggcaactgg

SEQ ID NO: 50 - DNA, 26 bp, Artificial Sequence
  primer
ggatccccgtcaccgacacctccaca

SEQ ID NO: 51 - DNA, 25 bp, Artificial Sequence
  primer
acatcacgctggcagagtacctcaa

SEQ ID NO: 52 - DNA, 25 bp, Artificial Sequence
  primer
ttgaggtactctgccagcgtgatgt

SEQ ID NO: 53 - protein, 436 aa, Artificial Sequence
  ilvA_T381A+F383A
MSETYVSEKSPGVMASGAELIRAADIQTAQARISSVIAPTPLQYCPRLSEETGAEIYLKREDLQDVRSYKIRGALNSGAQLTQEQRDAGIVAASAGNHAQGVAYVCKSLGVQGRIYVPVQTPKQKRDRIMVHGGEFVSLVVTGNNFDEASAAAHEDAERTGATLIEPFDARNTVIGQGTVAAEILSQLTSMGKSADHVMVPVGGGGLLAGVVSYMADMAPRTAIVGIEPAGAASMQAALHNGGPITLETVDPFVDGAAVKRVGDLNYTIVEKNQGRVHMMSATEGAVCTEMLDLYQNEGIIAEPAGALSIAGLKEMSFAPGSVVVCIISGGNNDVLRYAEIAERSLVHRGLKHYFLVNFPQKPGQLRHFLEDILGPDDDIALAEYLKRNNRETGTALVGIHLSEASGLDSLLERMEESAIDSRRLEPGTPEYEYLT

SEQ ID NO: 54 - DNA, 1311 bp, Artificial Sequence
  ilvA_T381A+F383A_nt
atgagtgaaacatacgtgtctgagaaaagtccaggagtgatggctagcggagcggagctgattcgtgccgccgacattcaaacggcgcaggcacgaatttcctccgtcattgcaccaactccattgcagtattgccctcgtctttctgaggaaaccggagcggaaatctaccttaagcgtgaggatctgcaggatgttcgttcctacaagatccgcggtgcgctgaactctggagcgcagctcacccaagagcagcgcgatgcaggtatcgttgccgcatctgcaggtaaccatgcccagggcgtggcctatgtgtgcaagtccttgggcgttcagggacgcatctatgttcctgtgcagactccaaagcaaaagcgtgaccgcatcatggttcacggcggagagtttgtctccttggtggtcactggcaataacttcgacgaagcatcggctgcagcgcatgaagatgcagagcgcaccggcgcaacgctgatcgagcctttcgatgctcgcaacaccgtcatcggtcagggcaccgtggctgctgagatcttgtcgcagctgacttccatgggcaagagtgcagatcacgtgatggttccagtcggcggtggcggacttcttgcaggtgtggtcagctacatggctgatatggcacctcgcactgcgatcgttggtatcgaaccagcgggagcagcatccatgcaggctgcattgcacaatggtggaccaatcactttggagactgttgatccctttgtggacggcgcagcagtcaaacgtgtcggagatctcaactacaccatcgtggagaagaaccagggtcgcgtgcacatgatgagcgcgaccgagggcgctgtgtgtactgagatgctcgatctttaccaaaacgaaggcatcatcgcggagcctgctggcgcgctgtctatcgctgggttgaaggaaatgtcctttgcacctggttctgtcgtggtgtgcatcatctctggtggcaacaacgatgtgctgcgttatgcggaaatcgctgagcgctccttggtgcaccgcggtttgaagcactacttcttggtgaacttcccgcaaaagcctggtcagttgcgtcacttcctggaagatatcctgggaccggatgatgacatcgcgctggcagagtacctcaagcgcaacaaccgtgagaccggtactgcgttggtgggtattcacttgagtgaagcatcaggattggattctttgctggaacgtatggaggaatcggcaattgattcccgtcgcctcgagccgggcacccctgagtacgaatacttgacctaa

SEQ ID NO: 55 - DNA, 22 bp, Artificial Sequence
  primer
aacacgaccggcatcccgtcgc

SEQ ID NO: 56 - DNA, 23 bp, Artificial Sequence
  primer
aaatcatttgagaaaactcgagg

SEQ ID NO: 57 - DNA, 45 bp, Artificial Sequence
  primer
gtgaattcgagctcggtacccaaatcatttgagaaaactcgaggc

SEQ ID NO: 58 - DNA, 45 bp, Artificial Sequence
  primer
ggtgatcatctcaacggtggaacacaggttgatgatcattgggtt

SEQ ID NO: 59 - DNA, 45 bp, Artificial Sequence
  primer
aacccaatgatcatcaacctgtgttccaccgttgagatgatcacc

SEQ ID NO: 60 - DNA, 42 bp, Artificial Sequence
  primer
ggtcgactctagaggatccccaagaaggcaacatcggacagc

SEQ ID NO: 61 - DNA, 21 bp, Artificial Sequence
  primer
atccattcaatggagtctgcg

SEQ ID NO: 62 - protein, 616 aa, Artificial Sequence
  leuA_P247C+R558H+G561D
MSPNDAFISAPAKIETPVGPRNEGQPAWNKQRGSSMPVNRYMPFEVEVEDISLPDRTWPDKKITVAPQWCAVDLRDGNQALIDPMSPERKRRMFELLVQMGFKEIEVGFPSASQTDFDFVREIIEKGMIPDDVTIQVLVQAREHLIRRTFEACEGAKNVIVHFYNSTSILQRNVVFRMDKVQVKKLATDAAELIKTIAQDYPDTNWRWQYSPESFTGTEVEYAKEVVDAVVEVMDPTPENPMIINLCSTVEMITPNVYADSIEWMHRNLNRRDSIILSLHPHNDRGTGVGAAELGYMAGADRIEGCLFGNGERTGNVCLVTLALNMLTQGVDPQLDFTDIRQIRSTVEYCNQLRVPERHPYGGDLVFTAFSGSHQDAVNKGLDAMAAKVQPGASSTEVSWEQLRDTEWEVPYLPIDPKDVGRDYEAVIRVNSQSGKGGVAYIMKTDHGLQIPRSMQVEFSTVVQNVTDAEGGEVNSKAMWDIFATEYLERTAPVEQIALRVENAQTENEDASITAELIHNGKDVTVDGRGNGPLAAYANALEKLGIDVEIQEYNQHAHTSDDDAEAAAYVLAEVNGRKVWGVGIAGSITYASLKAVTSAVNRALDVNHEAVLAGGV

SEQ ID NO: 63 - DNA, 1851 bp, Artificial Sequence
  leuA_P247C+R558H+G561D_nt
atgtctcctaacgatgcattcatctccgcacctgccaagatcgaaaccccagttgggcctcgcaacgaaggccagccagcatggaataagcagcgtggctcctcaatgccagttaaccgctacatgcctttcgaggttgaggtagaagatatttctctgccggaccgcacttggccagataaaaaaatcaccgttgcacctcagtggtgtgctgttgacctgcgtgacggcaaccaggctctgattgatccgatgtctcctgagcgtaagcgccgcatgtttgagctgctggttcagatgggcttcaaagaaatcgaggtcggtttcccttcagcttcccagactgattttgatttcgttcgtgagatcatcgaaaagggcatgatccctgacgatgtcaccattcaggttctggttcaggctcgtgagcacctgattcgccgtacttttgaagcttgcgaaggcgcaaaaaacgttatcgtgcacttctacaactccacctccatcctgcagcgcaacgtggtgttccgcatggacaaggtgcaggtgaagaagctggctaccgatgccgctgaactaatcaagaccatcgctcaggattacccagacaccaactggcgctggcagtactcccctgagtccttcaccggcactgaggttgagtacgccaaggaagttgtggacgcagttgttgaggtcatggatccaactcctgagaacccaatgatcatcaacctgtgttccaccgttgagatgatcacccctaacgtttacgcagactccattgaatggatgcaccgcaatctaaaccgtcgtgattccattatcctgtccctgcacccgcacaatgaccgtggcaccggcgttggcgcagctgagctgggctacatggctggcgctgaccgcatcgaaggctgcctgttcggcaacggcgagcgcaccggcaacgtctgcctggtcaccctggcactgaacatgctgacccagggcgttgaccctcagctggacttcaccgatatacgccagatccgcagcaccgttgaatactgcaaccagctgcgcgttcctgagcgccacccatacggcggtgacctggtcttcaccgctttctccggttcccaccaggacgctgtgaacaagggtctggacgccatggctgccaaggttcagccaggtgctagctccactgaagtttcttgggagcagctgcgcgacaccgaatgggaggttccttacctgcctatcgatccaaaggatgtcggtcgcgactacgaggctgttatccgcgtgaactcccagtccggcaagggcggcgttgcttacatcatgaagaccgatcacggtctgcagatccctcgctccatgcaggttgagttctccaccgttgtccagaacgtcaccgacgctgagggcggcgaggtcaactccaaggcaatgtgggatatcttcgccaccgagtacctggagcgcaccgcaccagttgagcagatcgcgctgcgcgtcgagaacgctcagaccgaaaacgaggatgcatccatcaccgccgagctcatccacaacggcaaggacgtcaccgtcgatggccgcggcaacggcccactggccgcttacgccaacgcgctggagaagctgggcatcgacgttgagatccaggaatacaaccagcacgcccacacctcggatgacgatgcagaagcagccgcctacgtgctggctgaggtcaacggccgcaaggtctggggcgtcggcatcgctggctccatcacctacgcttcgctgaaggcagtgacctccgccgtaaaccgcgcgctggacgtcaaccacgaggcagtcctggctggcggcgtttaa